European Patent Specification EP 3 548 096 B1, published November 20, 2024. Title: INHIBITOR-FUNCTIONALIZED ULTRASMALL NANOPARTICLES AND METHODS THEREOF. Applicant: MEMORIAL SLOAN KETTERING CANCER CENTER CORNELL UNIVERSITY THE CURATORS OF THE UNIVERSITY OF MISSOURI. The sequence listing filed with the application follows.

SEQUENCE LISTING (2 sequences)

SEQ ID NO: 1 - protein, 4 aa, Artificial Sequence
  source: /note="Description of Artificial Sequence: Synthetic peptide"
  MISC_FEATURE (1)..(4): /note="Cyclic"
RGDY

SEQ ID NO: 2 - protein, 9 aa, Artificial Sequence
  source: /note="Description of Artificial Sequence: Synthetic peptide"
  source: /note="N-term 4-amino-1-carboxy-methyl-piperidine modified"
  MOD_RES (8)..(8): Statine
HQWAVGHXL